European Patent Application EP 4 338 598 A1, published March 20, 2024. Title: Mass production method of flavoring agent with taste similar to sugar with D-allulose functionality. Applicant: NATIONAL UNIVERSITY CORPORATION KAGAWA UNIVERSIT. The sequence listing filed with the application follows.

SEQUENCE LISTING (1 sequence)

SEQ ID NO: 1 - protein, 289 aa, Arthrobacter histidinolovorans
MKIGCHGLVWTGRFDAEGIRYSVQKTKEAGFDLIEFPLMDPFSFDVATAKSALAEHGLTASASLGLSEATDVSSEDPAIVKAGEELLNRALDVLAELGATDFCGVIYSAMKKYMEPATEQGLSNSKAAIGRVVDRAAGLGINVSLEVVNRYETNVLNTGRQALSYLSDVKRPNLGVHLDTYHMNIEESDMFSPVLDTAEVLKYVHIGESHRGYLGTGNVDFDNFFKALGRIGYDGPVVFESFSSAVVAPDLSRMLGIWRNLWADNEELGAHANAFIRDKLTAIKTIELH